European Patent Specification EP 3 549 954 B1, published July 3, 2024. Title: High-Affinity TCR For NY-ESO. Applicant: GUANGDONG XIANGXUE LIFE SCIENCES, LTD. The sequence listing filed with the application follows.

SEQUENCE LISTING (104 sequences)

SEQ ID NO: 1 - protein, 109 aa, Artificial sequence
SQQGEEDPQALSIQEGENATMNCSYKTSINNLQWYRQNSGRGLVHLILIRSNEREKHSGRLRVTLDTSKKSSSLLITASRAADTASYFCATDANGKIIFGKGTRLHILP

SEQ ID NO: 2 - protein, 112 aa, Artificial sequence
DAGVIQSPRHEVTEMGQEVTLRCKPISGHDYLFWYRQTMMRGLELLIYFNNNVPIDDSGMPEDRFSAKMPNASFSTLKIQPSEPRDSAVYFCASSLGSNEQYFGPGTRLTVT

SEQ ID NO: 3 - protein, 109 aa, Artificial sequence
SQQGEEDPQALSIQEGENVTINCSYKTSINNLQWYRQNSGRGLVHLILIRSNEREKHSGRLRVTLDTSKKSSSLEITAVRPADTASYFCATDANGKIIFGKGTRLHILP

SEQ ID NO: 4 - protein, 112 aa, Artificial sequence
DAGVTQSPRHESVEMGQEVTLRCKPISGHDYLFWYRQTPKRGLELLIYFNNNVPIDDSGMPEDRFSAKMPNASFSTLKIQPVEPRDSAVYFCASSLGSNEQYFGPGTRLTVT

SEQ ID NO: 5 - DNA, 327 bp, Artificial sequence
tctcaacaaggtgaagaagatccgcaggccctgagtattcaagaaggtgaaaatgtgaccatcaactgctcttacaaaacgagtatcaacaatctgcagtggtaccgtcaaaattctggccgcggtctggttcatctgattctgatccgttccaacgaacgcgaaaaacactcaggccgtctgcgcgttaccctggataccagcaaaaaatcttctagtctggaaatcaccgcagtccgtccggcagatacggcaagctatttttgtgcaaccgacgctaatggtaaaattatcttcggcaaaggtacccgcctgcatattctgccg

SEQ ID NO: 6 - DNA, 336 bp, Artificial sequence
gatgcgggtgtcacgcagtctccgcgtcatgaaagtgtggaaatgggccaagaagttacgctgcgctgcaaaccgatcagcggtcacgactacctgttttggtaccgtcagaccccgaaacgcggcctggaactgctgatctacttcaacaataacgttccgattgatgactcgggtatgccggaagatcgttttagcgcgaaaatgccgaatgcctcgttcagcacgctgaaaattcagccggtcgaaccgcgtgactccgcagtgtatttttgtgcttcctcactgggcagtaacgaacagtacttcggcccgggtacccgtctgaccgtgacg

SEQ ID NO: 7 - protein, 24 aa, Artificial sequence
GGGSEGGGSEGGGSEGGGSEGGTG

SEQ ID NO: 8 - DNA, 72 bp, Artificial sequence
ggcggtggctccgaaggtggcggttcagaaggcggtggctcggaaggtggcggtagcgaaggcggtaccggt

SEQ ID NO: 9 - protein, 109 aa, Artificial sequence
SQQGEEDPQALSIQEGENVTINCSYKTSINNLQWYRQNSGRGLVHLILIRSNEREKHSGRLRVTLDTSKKSSSLEITAVRPADTASYFCATDAFAWWIFGKGTRLHILP

SEQ ID NO: 10 - protein, 109 aa, Artificial sequence
SQQGEEDPQALSIQEGENVTINCSYKGWAQNLQWYRQNSGRGLVHLILIRTGEQEKHSGRLRVTLDTSKKSSSLEITAVRPADTASYFCATDANARWNFGKGTRLHILP

SEQ ID NO: 11 - protein, 109 aa, Artificial sequence
SQQGEEDPQALSIQEGENVTINCSYKGSIQNLQWYRQNSGRGLVHLILIRTGEQEKHSGRLRVTLDTSKKSSSLEITAVRPADTASYFCATDANARWEFGKGTRLHILP

SEQ ID NO: 12 - protein, 109 aa, Artificial sequence
SQQGEEDPQALSIQEGENVTINCSYKGSIQNLQWYRQNSGRGLVHLILIRTGEQEKHSGRLRVTLDTSKKSSSLEITAVRPADTASYFCATDANARWDFGKGTRLHILP

SEQ ID NO: 13 - protein, 109 aa, Artificial sequence
SQQGEEDPQALSIQEGENVTINCSYKGWAQNLQWYRQNSGRGLVHLILIRSNEREKHSGRLRVTLDTSKKSSSLEITAVRPADTASYFCATDANARWNFGKGTRLHILP

SEQ ID NO: 14 - protein, 109 aa, Artificial sequence
SQQGEEDPQALSIQEGENVTINCSYKGWVQNLQWYRQNSGRGLVHLILIRTGEQEKHSGRLRVTLDTSKKSSSLEITAVRPADTASYFCATDANARWDFGKGTRLHILP

SEQ ID NO: 15 - protein, 109 aa, Artificial sequence
SQQGEEDPQALSIQEGENVTINCSYKGSIQNLQWYRQNSGRGLVHLILIRSNEREKHSGRLRVTLDTSKKSSSLEITAVRPADTASYFCATDANARWDFGKGTRLHILP

SEQ ID NO: 16 - protein, 105 aa, Artificial sequence
SQQGEEDPQALSIQEGENVTINCSYKGWAQNRQNSGRGLVHLILIRSNEREKHSGRLRVTLDTSKKSSSLEITAVRPADTASYFCATDANARWDFGKGTRLHILP

SEQ ID NO: 17 - protein, 109 aa, Artificial sequence
SQQGEEDPQALSIQEGENVTINCSYKGSIQNLQWYRQNSGRGLVHLILIRSNEREKHSGRLRVTLDTSKKSSSLEITAVRPADTASYFCATDANARWEFGKGTRLHILP

SEQ ID NO: 18 - protein, 109 aa, Artificial sequence
SQQGEEDPQALSIQEGENVTINCSYKTSINNLQWYRQNSGRGLVHLILIRSNEREKHSGRLRVTLDTSKKSSSLEITAVRPADTASYFCMYDENGKIIFGKGTRLHILP

SEQ ID NO: 19 - protein, 109 aa, Artificial sequence
SQQGEEDPQALSIQEGENVTINCSYKTSINNLQWYRQNSGRGLVHLILIRSNEREKHSGRLRVTLDTSKKSSSLEITAVRPADTASYFCMYDQNGKIIFGKGTRLHILP

SEQ ID NO: 20 - protein, 109 aa, Artificial sequence
SQQGEEDPQALSIQEGENVTINCSYKTSINNLQWYRQNSGRGLVHLILIRSNEREKHSGRLRVTLDTSKKSSSLEITAVRPADTASYFCATDAYGTVQFGKGTRLHILP

SEQ ID NO: 21 - protein, 109 aa, Artificial sequence
SQQGEEDPQALSIQEGENVTINCSYKTSINNLQWYRQNSGRGLVHLILIRSNEREKHSGRLRVTLDTSKKSSSLEITAVRPADTASYFCATDANGTVQFGKGTRLHILP

SEQ ID NO: 22 - protein, 109 aa, Artificial sequence
SQQGEEDPQALSIQEGENVTINCSYKTSINNLQWYRQNSGRGLVHLILIRSNEREKHSGRLRVTLDTSKKSSSLEITAVRPADTASYFCATDANGSVQFGKGTRLHILP

SEQ ID NO: 23 - protein, 109 aa, Artificial sequence
SQQGEEDPQALSIQEGENVTINCSYKTSINNLQWYRQNSGRGLVHLILIRSNEREKHSGRLRVTLDTSKKSSSLEITAVRPADTASYFCATDAYGRYIFGKGTRLHILP

SEQ ID NO: 24 - protein, 109 aa, Artificial sequence
SQQGEEDPQALSIQEGENVTINCSYKTSINNLQWYRQNSGRGLVHLILIRSNEREKHSGRLRVTLDTSKKSSSLEITAVRPADTASYFCATDANQMWKFGKGTRLHILP

SEQ ID NO: 25 - protein, 109 aa, Artificial sequence
SQQGEEDPQALSIQEGENVTINCSYKTSINNLQWYRQNSGRGLVHLILIRSNEREKHSGRLRVTLDTSKKSSSLEITAVRPADTASYFCATDAYGLPIFGKGTRLHILP

SEQ ID NO: 26 - protein, 109 aa, Artificial sequence
SQQGEEDPQALSIQEGENVTINCSYKTSINNLQWYRQNSGRGLVHLILIRSNEREKHSGRLRVTLDTSKKSSSLEITAVRPADTASYFCATDANGLPVFGKGTRLHILP

SEQ ID NO: 27 - protein, 109 aa, Artificial sequence
SQQGEEDPQALSIQEGENVTINCSYKTSINNLQWYRQNSGRGLVHLILIRSNEREKHSGRLRVTLDTSKKSSSLEITAVRPADTASYFCATDANGRWEFGKGTRLHILP

SEQ ID NO: 28 - protein, 109 aa, Artificial sequence
SQQGEEDPQALSIQEGENVTINCSYKTSINNLQWYRQNSGRGLVHLILIRSNEREKHSGRLRVTLDTSKKSSSLEITAVRPADTASYFCATDANGTVGFGKGTRLHILP

SEQ ID NO: 29 - protein, 109 aa, Artificial sequence
SQQGEEDPQALSIQEGENVTINCSYKTSINNLQWYRQNSGRGLVHLILIRSNEREKHSGRLRVTLDTSKKSSSLEITAVRPADTASYFCATDANGRWMFGKGTRLHILP

SEQ ID NO: 30 - protein, 109 aa, Artificial sequence
SQQGEEDPQALSIQEGENVTINCSYKTSINNLQWYRQNSGRGLVHLILIRSNEREKHSGRLRVTLDTSKKSSSLEITAVRPADTASYFCATDANGLWSFGKGTRLHILP

SEQ ID NO: 31 - protein, 109 aa, Artificial sequence
SQQGEEDPQALSIQEGENVTINCSYKGWAQNLQWYRQNSGRGLVHLILIRTGEQEKHSGRLRVTLDTSKKSSSLEITAVRPADTASYFCATDANARWDFGKGTRLHILP

SEQ ID NO: 32 - protein, 109 aa, Artificial sequence
SQQGEEDPQALSIQEGENVTINCSYKGWAQNLQWYRQNSGRGLVHLILIRTGQAEKHSGRLRVTLDTSKKSSSLEITAVRPADTASYFCATDANARWEFGKGTRLHILP

SEQ ID NO: 33 - protein, 109 aa, Artificial sequence
SQQGEEDPQALSIQEGENVTINCSYKGSIQNLQWYRQNSGRGLVHLILIRSNEREKHSGRLRVTLDTSKKSSSLEITAVRPADTASYFCATDAFAWWIFGKGTRLHILP

SEQ ID NO: 34 - protein, 109 aa, Artificial sequence
SQQGEEDPQALSIQEGENVTINCSYKGWVQNLQWYRQNSGRGLVHLILIRTGEQEKHSGRLRVTLDTSKKSSSLEITAVRPADTASYFCATDANARWNFGKGTRLHILP

SEQ ID NO: 35 - protein, 109 aa, Artificial sequence
SQQGEEDPQALSIQEGENVTINCSYKGSIQNLQWYRQNSGRGLVHLILIRTGEQEKHSGRLRVTLDTSKKSSSLEITAVRPADTASYFCATDAWARWIFGKGTRLHILP

SEQ ID NO: 36 - protein, 109 aa, Artificial sequence
SQQGEEDPQALSIQEGENVTINCSYKGWVQNLQWYRQNSGRGLVHLILIRTGQAEKHSGRLRVTLDTSKKSSSLEITAVRPADTASYFCATDANARWEFGKGTRLHILP

SEQ ID NO: 37 - protein, 109 aa, Artificial sequence
SQQGEEDPQALSIQEGENVTINCSYKGSIQNLQWYRQNSGRGLVHLILIRTGEQEKHSGRLRVTLDTSKKSSSLEITAVRPADTASYFCATDANARWNFGKGTRLHILP

SEQ ID NO: 38 - protein, 112 aa, Artificial sequence
DAGVTQSPRHESVEMGQEVTLRCKPISGHDYLFWYRQTPKRGLELLIYFNHGAVIDDSGMPEDRFSAKMPNASFSTLKIQPVEPRDSAVYFCASSLGSNEQYFGPGTRLTVT

SEQ ID NO: 39 - protein, 112 aa, Artificial sequence
DAGVTQSPRHESVEMGQEVTLRCKPISGHDYLFWYRQTPKRGLELLIYFNHGAVIDDSGMPEDRFSAKMPNASFSTLKIQPVEPRDSAVYFCASQRGSNEQYFGPGTRLTVT

SEQ ID NO: 40 - protein, 112 aa, Artificial sequence
DAGVTQSPRHESVEMGQEVTLRCKPISGHDYLFWYRQTPKRGLELLIYFNHGAVIDDSGMPEDRFSAKMPNASFSTLKIQPVEPRDSAVYFCASQKGANEQYFGPGTRLTVT

SEQ ID NO: 41 - protein, 112 aa, Artificial sequence
DAGVTQSPRHESVEMGQEVTLRCKPISGHDYLFWYRQTPKRGLELLIYFNHGAVIDDSGMPEDRFSAKMPNASFSTLKIQPVEPRDSAVYFCASQLGSNEQYFGPGTRLTVT

SEQ ID NO: 42 - protein, 112 aa, Artificial sequence
DAGVTQSPRHESVEMGQEVTLRCKPISGHDYLFWYRQTPKRGLELLIYFNHGAVIDDSGMPEDRFSAKMPNASFSTLKIQPVEPRDSAVYFCASQLGANEQYFGPGTRLTVT

SEQ ID NO: 43 - protein, 112 aa, Artificial sequence
DAGVTQSPRHESVEMGQEVTLRCKPISGHDYLFWYRQTPKRGLELLIYFNNNVPIDDSGMPEDRFSAKMPNASFSTLKIQPVEPRDSAVYFCASQLGGNEQYFGPGTRLTVT

SEQ ID NO: 44 - protein, 112 aa, Artificial sequence
DAGVTQSPRHESVEMGQEVTLRCKPISGHDYLFWYRQTPKRGLELLIYFNNNVPIDDSGMPEDRFSAKMPNASFSTLKIQPVEPRDSAVYFCASQKGANEQYFGPGTRLTVT

SEQ ID NO: 45 - protein, 112 aa, Artificial sequence
DAGVTQSPRHESVEMGQEVTLRCKPISGHDYLFWYRQTPKRGLELLIYFNNNVPIDDSGMPEDRFSAKMPNASFSTLKIQPVEPRDSAVYFCASQLGPNEQYFGPGTRLTVT

SEQ ID NO: 46 - protein, 112 aa, Artificial sequence
DAGVTQSPRHESVEMGQEVTLRCKPISGHDYLFWYRQTPKRGLELLIYFNNNVPIDDSGMPEDRFSAKMPNASFSTLKIQPVEPRDSAVYFCASQRGANEQYFGPGTRLTVT

SEQ ID NO: 47 - protein, 112 aa, Artificial sequence
DAGVTQSPRHESVEMGQEVTLRCKPISGHDYLFWYRQTPKRGLELLIYFNNNVPIDDSGMPEDRFSAKMPNASFSTLKIQPVEPRDSAVYFCASQMGSNEQYFGPGTRLTVT

SEQ ID NO: 48 - protein, 112 aa, Artificial sequence
DAGVTQSPRHESVEMGQEVTLRCKPISGHDYLFWYRQTPKRGLELLIYFNNNVPIDDSGMPEDRFSAKMPNASFSTLKIQPVEPRDSAVYFCASQLGSNEQYFGPGTRLTVT

SEQ ID NO: 49 - protein, 112 aa, Artificial sequence
DAGVTQSPRHESVEMGQEVTLRCKPISGHDYLFWYRQTPKRGLELLIYFNNNVPIDDSGMPEDRFSAKMPNASFSTLKIQPVEPRDSAVYFCASQLGANEQYFGPGTRLTVT

SEQ ID NO: 50 - protein, 112 aa, Artificial sequence; identical to SEQ ID NO: 47

SEQ ID NO: 51 - protein, 112 aa, Artificial sequence
DAGVTQSPRHESVEMGQEVTLRCKPISGHDYLFWYRQTPKRGLELLIYFNNNVPIDDSGMPEDRFSAKMPNASFSTLKIQPVEPRDSAVYFCASQRGSNEQYFGPGTRLTVT

SEQ ID NO: 52 - protein, 112 aa, Artificial sequence
DAGVTQSPRHESVEMGQEVTLRCKPISGHDYLFWYRQTPKRGLELLIYFNNNVPIDDSGMPEDRFSAKMPNASFSTLKIQPVEPRDSAVYFCASQMGANEQYFGPGTRLTVT

SEQ ID NO: 53 - protein, 112 aa, Artificial sequence
DAGVTQSPRHESVEMGQEVTLRCKPISGHDYLFWYRQTPKRGLELLIYFNNNVPIDDSGMPEDRFSAKMPNASFSTLKIQPVEPRDSAVYFCASMLGSNEQYFGPGTRLTVT

SEQ ID NO: 54 - protein, 245 aa, Artificial sequence
SQQGEEDPQALSIQEGENVTINCSYKTSINNLQWYRQNSGRGLVHLILIRSNEREKHSGRLRVTLDTSKKSSSLEITAVRPADTASYFCATDANGKIIFGKGTRLHILPGGGSEGGGSEGGGSEGGGSEGGTGDAGVTQSPRHESVEMGQEVTLRCKPISGHDYLFWYRQTPKRGLELLIYFNNNVPIDDSGMPEDRFSAKMPNASFSTLKIQPVEPRDSAVYFCASSLGSNEQYFGPGTRLTVT

SEQ ID NO: 55 - DNA, 735 bp, Artificial sequence
tctcaacaaggtgaagaagatccgcaggccctgagtattcaagaaggtgaaaatgtgaccatcaactgctcttacaaaacgagtatcaacaatctgcagtggtaccgtcaaaattctggccgcggtctggttcatctgattctgatccgttccaacgaacgcgaaaaacactcaggccgtctgcgcgttaccctggataccagcaaaaaatcttctagtctggaaatcaccgcagtccgtccggcagatacggcaagctatttttgtgcaaccgacgctaatggtaaaattatcttcggcaaaggtacccgcctgcatattctgccgggcggtggctccgaaggtggcggttcagaaggcggtggctcggaaggtggcggtagcgaaggcggtaccggtgatgcgggtgtcacgcagtctccgcgtcatgaaagtgtggaaatgggccaagaagttacgctgcgctgcaaaccgatcagcggtcacgactacctgttttggtaccgtcagaccccgaaacgcggcctggaactgctgatctacttcaacaataacgttccgattgatgactcgggtatgccggaagatcgttttagcgcgaaaatgccgaatgcctcgttcagcacgctgaaaattcagccggtcgaaccgcgtgactccgcagtgtatttttgtgcttcctcactgggcagtaacgaacagtacttcggcccgggtacccgtctgaccgtgacg

SEQ ID NO: 56 - protein, 203 aa, Artificial sequence
SQQGEEDPQALSIQEGENATMNCSYKTSINNLQWYRQNSGRGLVHLILIRSNEREKHSGRLRVTLDTSKKSSSLLITASRAADTASYFCATDANGKIIFGKGTRLHILPNIQNPDPAVYQLRDSKSSDKSVCLFTDFDSQTNVSQSKDSDVYITDKCVLDMRSMDFKSNSAVAWSNKSDFACANAFNNSIIPEDTFFPSPESS

SEQ ID NO: 57 - protein, 242 aa, Artificial sequence
DAGVIQSPRHEVTEMGQEVTLRCKPISGHDYLFWYRQTMMRGLELLIYFNNNVPIDDSGMPEDRFSAKMPNASFSTLKIQPSEPRDSAVYFCASSLGSNEQYFGPGTRLTVTEDLKNVFPPEVAVFEPSEAEISHTQKATLVCLATGFYPDHVELSWWVNGKEVHSGVCTDPQPLKEQPALNDSRYALSSRLRVSATFWQDPRNHFRCQVQFYGLSENDEWTQDRAKPVTQIVSAEAWGRAD

SEQ ID NO: 58 - protein, 109 aa, Artificial sequence
SQQGEEDPQALSIQEGENATMNCSYKTSINNLQWYRQNSGRGLVHLILIRSNEREKHSGRLRVTLDTSKKSSSLLITASRAADTASYFCATDAFAWWIFGKGTRLHILP

SEQ ID NO: 59 - protein, 109 aa, Artificial sequence
SQQGEEDPQALSIQEGENATMNCSYKGWAQNLQWYRQNSGRGLVHLILIRTGEQEKHSGRLRVTLDTSKKSSSLLITASRAADTASYFCATDANARWNFGKGTRLHILP

SEQ ID NO: 60 - protein, 109 aa, Artificial sequence
SQQGEEDPQALSIQEGENATMNCSYKGSIQNLQWYRQNSGRGLVHLILIRTGEQEKHSGRLRVTLDTSKKSSSLLITASRAADTASYFCATDANARWEFGKGTRLHILP

SEQ ID NO: 61 - protein, 109 aa, Artificial sequence
SQQGEEDPQALSIQEGENATMNCSYKGSIQNLQWYRQNSGRGLVHLILIRTGEQEKHSGRLRVTLDTSKKSSSLLITASRAADTASYFCATDANARWDFGKGTRLHILP

SEQ ID NO: 62 - protein, 109 aa, Artificial sequence
SQQGEEDPQALSIQEGENATMNCSYKGWAQNLQWYRQNSGRGLVHLILIRSNEREKHSGRLRVTLDTSKKSSSLLITASRAADTASYFCATDANARWNFGKGTRLHILP

SEQ ID NO: 63 - protein, 109 aa, Artificial sequence
SQQGEEDPQALSIQEGENATMNCSYKGWVQNLQWYRQNSGRGLVHLILIRTGEQEKHSGRLRVTLDTSKKSSSLLITASRAADTASYFCATDANARWDFGKGTRLHILP

SEQ ID NO: 64 - protein, 109 aa, Artificial sequence
SQQGEEDPQALSIQEGENATMNCSYKGSIQNLQWYRQNSGRGLVHLILIRSNEREKHSGRLRVTLDTSKKSSSLLITASRAADTASYFCATDANARWDFGKGTRLHILP

SEQ ID NO: 65 - protein, 105 aa, Artificial sequence
SQQGEEDPQALSIQEGENATMNCSYKGWAQNRQNSGRGLVHLILIRSNEREKHSGRLRVTLDTSKKSSSLLITASRAADTASYFCATDANARWDFGKGTRLHILP

SEQ ID NO: 66 - protein, 109 aa, Artificial sequence
SQQGEEDPQALSIQEGENATMNCSYKGSIQNLQWYRQNSGRGLVHLILIRSNEREKHSGRLRVTLDTSKKSSSLLITASRAADTASYFCATDANARWEFGKGTRLHILP

SEQ ID NO: 67 - protein, 109 aa, Artificial sequence
SQQGEEDPQALSIQEGENATMNCSYKTSINNLQWYRQNSGRGLVHLILIRSNEREKHSGRLRVTLDTSKKSSSLLITASRAADTASYFCMYDENGKIIFGKGTRLHILP

SEQ ID NO: 68 - protein, 109 aa, Artificial sequence
SQQGEEDPQALSIQEGENATMNCSYKTSINNLQWYRQNSGRGLVHLILIRSNEREKHSGRLRVTLDTSKKSSSLLITASRAADTASYFCMYDQNGKIIFGKGTRLHILP

SEQ ID NO: 69 - protein, 109 aa, Artificial sequence
SQQGEEDPQALSIQEGENATMNCSYKTSINNLQWYRQNSGRGLVHLILIRSNEREKHSGRLRVTLDTSKKSSSLLITASRAADTASYFCATDAYGTVQFGKGTRLHILP

SEQ ID NO: 70 - protein, 109 aa, Artificial sequence
SQQGEEDPQALSIQEGENATMNCSYKTSINNLQWYRQNSGRGLVHLILIRSNEREKHSGRLRVTLDTSKKSSSLLITASRAADTASYFCATDANGTVQFGKGTRLHILP

SEQ ID NO: 71 - protein, 109 aa, Artificial sequence
SQQGEEDPQALSIQEGENATMNCSYKTSINNLQWYRQNSGRGLVHLILIRSNEREKHSGRLRVTLDTSKKSSSLLITASRAADTASYFCATDANGSVQFGKGTRLHILP

SEQ ID NO: 72 - protein, 109 aa, Artificial sequence
SQQGEEDPQALSIQEGENATMNCSYKTSINNLQWYRQNSGRGLVHLILIRSNEREKHSGRLRVTLDTSKKSSSLLITASRAADTASYFCATDAYGRYIFGKGTRLHILP

SEQ ID NO: 73 - protein, 109 aa, Artificial sequence
SQQGEEDPQALSIQEGENATMNCSYKTSINNLQWYRQNSGRGLVHLILIRSNEREKHSGRLRVTLDTSKKSSSLLITASRAADTASYFCATDANQMWKFGKGTRLHILP

SEQ ID NO: 74 - protein, 109 aa, Artificial sequence
SQQGEEDPQALSIQEGENATMNCSYKTSINNLQWYRQNSGRGLVHLILIRSNEREKHSGRLRVTLDTSKKSSSLLITASRAADTASYFCATDAYGLPIFGKGTRLHILP

SEQ ID NO: 75 - protein, 109 aa, Artificial sequence
SQQGEEDPQALSIQEGENATMNCSYKTSINNLQWYRQNSGRGLVHLILIRSNEREKHSGRLRVTLDTSKKSSSLLITASRAADTASYFCATDANGLPVFGKGTRLHILP

SEQ ID NO: 76 - protein, 109 aa, Artificial sequence
SQQGEEDPQALSIQEGENATMNCSYKTSINNLQWYRQNSGRGLVHLILIRSNEREKHSGRLRVTLDTSKKSSSLLITASRAADTASYFCATDANGRWEFGKGTRLHILP

SEQ ID NO: 77 - protein, 109 aa, Artificial sequence
SQQGEEDPQALSIQEGENATMNCSYKTSINNLQWYRQNSGRGLVHLILIRSNEREKHSGRLRVTLDTSKKSSSLLITASRAADTASYFCATDANGTVGFGKGTRLHILP

SEQ ID NO: 78 - protein, 109 aa, Artificial sequence
SQQGEEDPQALSIQEGENATMNCSYKTSINNLQWYRQNSGRGLVHLILIRSNEREKHSGRLRVTLDTSKKSSSLLITASRAADTASYFCATDANGRWMFGKGTRLHILP

SEQ ID NO: 79 - protein, 109 aa, Artificial sequence
SQQGEEDPQALSIQEGENATMNCSYKTSINNLQWYRQNSGRGLVHLILIRSNEREKHSGRLRVTLDTSKKSSSLLITASRAADTASYFCATDANGLWSFGKGTRLHILP

SEQ ID NO: 80 - protein, 109 aa, Artificial sequence
SQQGEEDPQALSIQEGENATMNCSYKGWAQNLQWYRQNSGRGLVHLILIRTGEQEKHSGRLRVTLDTSKKSSSLLITASRAADTASYFCATDANARWDFGKGTRLHILP

SEQ ID NO: 81 - protein, 109 aa, Artificial sequence
SQQGEEDPQALSIQEGENATMNCSYKGWAQNLQWYRQNSGRGLVHLILIRTGQAEKHSGRLRVTLDTSKKSSSLLITASRAADTASYFCATDANARWEFGKGTRLHILP

SEQ ID NO: 82 - protein, 109 aa, Artificial sequence
SQQGEEDPQALSIQEGENATMNCSYKGSIQNLQWYRQNSGRGLVHLILIRSNEREKHSGRLRVTLDTSKKSSSLLITASRAADTASYFCATDAFAWWIFGKGTRLHILP

SEQ ID NO: 83 - protein, 109 aa, Artificial sequence
SQQGEEDPQALSIQEGENATMNCSYKGWVQNLQWYRQNSGRGLVHLILIRTGEQEKHSGRLRVTLDTSKKSSSLLITASRAADTASYFCATDANARWNFGKGTRLHILP

SEQ ID NO: 84 - protein, 109 aa, Artificial sequence
SQQGEEDPQALSIQEGENATMNCSYKGSIQNLQWYRQNSGRGLVHLILIRTGEQEKHSGRLRVTLDTSKKSSSLLITASRAADTASYFCATDAWARWIFGKGTRLHILP

SEQ ID NO: 85 - protein, 109 aa, Artificial sequence
SQQGEEDPQALSIQEGENATMNCSYKGWVQNLQWYRQNSGRGLVHLILIRTGQAEKHSGRLRVTLDTSKKSSSLLITASRAADTASYFCATDANARWEFGKGTRLHILP

SEQ ID NO: 86 - protein, 109 aa, Artificial sequence
SQQGEEDPQALSIQEGENATMNCSYKGSIQNLQWYRQNSGRGLVHLILIRTGEQEKHSGRLRVTLDTSKKSSSLLITASRAADTASYFCATDANARWNFGKGTRLHILP

SEQ ID NO: 87 - protein, 112 aa, Artificial sequence
DAGVIQSPRHEVTEMGQEVTLRCKPISGHDYLFWYRQTMMRGLELLIYFNHGAVIDDSGMPEDRFSAKMPNASFSTLKIQPSEPRDSAVYFCASSLGSNEQYFGPGTRLTVT

SEQ ID NO: 88 - protein, 112 aa, Artificial sequence
DAGVIQSPRHEVTEMGQEVTLRCKPISGHDYLFWYRQTMMRGLELLIYFNHGAVIDDSGMPEDRFSAKMPNASFSTLKIQPSEPRDSAVYFCASQRGSNEQYFGPGTRLTVT

SEQ ID NO: 89 - protein, 112 aa, Artificial sequence
DAGVIQSPRHEVTEMGQEVTLRCKPISGHDYLFWYRQTMMRGLELLIYFNHGAVIDDSGMPEDRFSAKMPNASFSTLKIQPSEPRDSAVYFCASQKGANEQYFGPGTRLTVT

SEQ ID NO: 90 - protein, 112 aa, Artificial sequence
DAGVIQSPRHEVTEMGQEVTLRCKPISGHDYLFWYRQTMMRGLELLIYFNHGAVIDDSGMPEDRFSAKMPNASFSTLKIQPSEPRDSAVYFCASQLGSNEQYFGPGTRLTVT

SEQ ID NO: 91 - protein, 112 aa, Artificial sequence
DAGVIQSPRHEVTEMGQEVTLRCKPISGHDYLFWYRQTMMRGLELLIYFNHGAVIDDSGMPEDRFSAKMPNASFSTLKIQPSEPRDSAVYFCASQLGANEQYFGPGTRLTVT

SEQ ID NO: 92 - protein, 112 aa, Artificial sequence
DAGVIQSPRHEVTEMGQEVTLRCKPISGHDYLFWYRQTMMRGLELLIYFNNNVPIDDSGMPEDRFSAKMPNASFSTLKIQPSEPRDSAVYFCASQLGGNEQYFGPGTRLTVT

SEQ ID NO: 93 - protein, 112 aa, Artificial sequence
DAGVIQSPRHEVTEMGQEVTLRCKPISGHDYLFWYRQTMMRGLELLIYFNNNVPIDDSGMPEDRFSAKMPNASFSTLKIQPSEPRDSAVYFCASQKGANEQYFGPGTRLTVT

SEQ ID NO: 94 - protein, 112 aa, Artificial sequence
DAGVIQSPRHEVTEMGQEVTLRCKPISGHDYLFWYRQTMMRGLELLIYFNNNVPIDDSGMPEDRFSAKMPNASFSTLKIQPSEPRDSAVYFCASQLGPNEQYFGPGTRLTVT

SEQ ID NO: 95 - protein, 112 aa, Artificial sequence
DAGVIQSPRHEVTEMGQEVTLRCKPISGHDYLFWYRQTMMRGLELLIYFNNNVPIDDSGMPEDRFSAKMPNASFSTLKIQPSEPRDSAVYFCASQRGANEQYFGPGTRLTVT

SEQ ID NO: 96 - protein, 112 aa, Artificial sequence
DAGVIQSPRHEVTEMGQEVTLRCKPISGHDYLFWYRQTMMRGLELLIYFNNNVPIDDSGMPEDRFSAKMPNASFSTLKIQPSEPRDSAVYFCASQMGSNEQYFGPGTRLTVT

SEQ ID NO: 97 - protein, 112 aa, Artificial sequence
DAGVIQSPRHEVTEMGQEVTLRCKPISGHDYLFWYRQTMMRGLELLIYFNNNVPIDDSGMPEDRFSAKMPNASFSTLKIQPSEPRDSAVYFCASQLGSNEQYFGPGTRLTVT

SEQ ID NO: 98 - protein, 112 aa, Artificial sequence
DAGVIQSPRHEVTEMGQEVTLRCKPISGHDYLFWYRQTMMRGLELLIYFNNNVPIDDSGMPEDRFSAKMPNASFSTLKIQPSEPRDSAVYFCASQLGANEQYFGPGTRLTVT

SEQ ID NO: 99 - protein, 112 aa, Artificial sequence; identical to SEQ ID NO: 96

SEQ ID NO: 100 - protein, 112 aa, Artificial sequence
DAGVIQSPRHEVTEMGQEVTLRCKPISGHDYLFWYRQTMMRGLELLIYFNNNVPIDDSGMPEDRFSAKMPNASFSTLKIQPSEPRDSAVYFCASQRGSNEQYFGPGTRLTVT

SEQ ID NO: 101 - protein, 112 aa, Artificial sequence
DAGVIQSPRHEVTEMGQEVTLRCKPISGHDYLFWYRQTMMRGLELLIYFNNNVPIDDSGMPEDRFSAKMPNASFSTLKIQPSEPRDSAVYFCASQMGANEQYFGPGTRLTVT

SEQ ID NO: 102 - protein, 112 aa, Artificial sequence
DAGVIQSPRHEVTEMGQEVTLRCKPISGHDYLFWYRQTMMRGLELLIYFNNNVPIDDSGMPEDRFSAKMPNASFSTLKIQPSEPRDSAVYFCASMLGSNEQYFGPGTRLTVT

SEQ ID NO: 103 - protein, 203 aa, Artificial sequence
SQQGEEDPQALSIQEGENATMNCSYKTSINNLQWYRQNSGRGLVHLILIRSNEREKHSGRLRVTLDTSKKSSSLLITASRAADTASYFCATDANGKIIFGKGTRLHILPNIQNPDPAVYQLRDSKSSDKSVCLFTDFDSQTNVSQSKDSDVYITDKTVLDMRSMDFKSNSAVAWSNKSDFACANAFNNSIIPEDTFFPSPESS

SEQ ID NO: 104 - protein, 242 aa, Artificial sequence
DAGVIQSPRHEVTEMGQEVTLRCKPISGHDYLFWYRQTMMRGLELLIYFNNNVPIDDSGMPEDRFSAKMPNASFSTLKIQPSEPRDSAVYFCASSLGSNEQYFGPGTRLTVTEDLKNVFPPEVAVFEPSEAEISHTQKATLVCLATGFYPDHVELSWWVNGKEVHSGVSTDPQPLKEQPALNDSRYALSSRLRVSATFWQDPRNHFRCQVQFYGLSENDEWTQDRAKPVTQIVSAEAWGRAD